European Patent Specification EP 3 071 237 B1, published June 26, 2024. Title: Antibody-drug conjugate formulations. Applicant: Genmab A/S. The sequence listing filed with the application follows.

SEQUENCE LISTING (80 sequences)

SEQ ID NO: 1 - protein, 119 aa, homo sapiens
QVQLVESGGGVVQPGRSLRLSCVASGFTVSNDGMHWVRQAPGKGLEWVALIWYDGVNKNYADSVKGRFTISRDKSKNTLYLQMNSLRAEDTAVYYCARRPGTFYGLDVWGQGTTVTVSS

SEQ ID NO: 2 - protein, 8 aa, homo sapiens
GFTVSNDG

SEQ ID NO: 3 - protein, 8 aa, homo sapiens
IWYDGVNK

SEQ ID NO: 4 - protein, 12 aa, homo sapiens
ARRPGTFYGLDV

SEQ ID NO: 5 - protein, 118 aa, homo sapiens
EVQLLESGGGLVQPGGSLRLSCAASGFTFSNYAMSWVRQAPGKGLEWVSSISGSGDYTYYTDSVKGRFTISRDNSKNTLYLQMNSLRAEDTAVYYCARSPWGYYLDSWGQGTLVTVSS

SEQ ID NO: 6 - protein, 8 aa, homo sapiens
GFTFSNYA

SEQ ID NO: 7 - protein, 8 aa, homo sapiens
ISGSGDYT

SEQ ID NO: 8 - protein, 11 aa, homo sapiens
ARSPWGYYLDS

SEQ ID NO: 9 - protein, 120 aa, homo sapiens
EVQLLESGGGLVQPGGSLRLSCAASGFTFSSYAMSWVRQAPGKGLEWVSAISGSGDSTNYADSVKGRFTISRDNSKNTLYLQMNSLRAEDTAVYYCAKDGYFLLWYFDLWGRGTLVTVSS

SEQ ID NO: 10 - protein, 8 aa, homo sapiens
GFTFSSYA

SEQ ID NO: 11 - protein, 8 aa, homo sapiens
ISGSGDST

SEQ ID NO: 12 - protein, 13 aa, homo sapiens
AKDGYFLLWYFDL

SEQ ID NO: 13 - protein, 118 aa, homo sapiens
EVQLLESGGGLVQPGGSLRLSCAASGFTFSSYGMSWVRQAPGKGLEWVSVISGSGGTTYYADSVKGRFTISRDNSKNTLYLQMNSLRAEDTAVYYCAKAPWTYYFDYWGQGTLVTVSS

SEQ ID NO: 14 - protein, 8 aa, homo sapiens
GFTFSSYG

SEQ ID NO: 15 - protein, 8 aa, homo sapiens
ISGSGGTT

SEQ ID NO: 16 - protein, 11 aa, homo sapiens
AKAPWTYYFDY

SEQ ID NO: 17 - protein, 118 aa, homo sapiens
EVQLLESGGGLVQPGGSLRLSCAASGFTFNNYAMSWVRQAPGKGLEWVSSISGSGGRTYYADSVKGRFTISRDNSKNTLFLQMNSLRAEDTAVYYCAKTPWGYYFDYWGQGTLVTVSS

SEQ ID NO: 18 - protein, 8 aa, homo sapiens
GFTFNNYA

SEQ ID NO: 19 - protein, 8 aa, homo sapiens
ISGSGGRT

SEQ ID NO: 20 - protein, 11 aa, homo sapiens
AKTPWGYYFDY

SEQ ID NO: 21 - protein, 118 aa, homo sapiens
EVQLLESGGGLVQPGGSLRLSCAASGFTFSNYAMSWVRQAPAKGLDWVSGISGSGVTTYYADSVKGRFTISRDNSKDTLYLQMNSLRAEDTAVYFCAKTPWGYYFDYWGQGILVAVSS

SEQ ID NO: 22 - protein, 8 aa, homo sapiens
GFTFSNYA

SEQ ID NO: 23 - protein, 8 aa, homo sapiens
ISGSGVTT

SEQ ID NO: 24 - protein, 11 aa, homo sapiens
AKTPWGYYFDY

SEQ ID NO: 25 - protein, 120 aa, homo sapiens
QVQLVESGGGVVQPGRSLRLSCAASGFTFSRYAMHWVRQAPGKGLEWVAVISNDGYNDYYADSVKGRFTVSRDNSKNTLYLQMNSLRAEDTAVYYCARDGQLGRGYFDYWGQGTLVTVSS

SEQ ID NO: 26 - protein, 8 aa, homo sapiens
GFTFSRYA

SEQ ID NO: 27 - protein, 8 aa, homo sapiens
ISNDGYND

SEQ ID NO: 28 - protein, 13 aa, homo sapiens
ARDGQLGRGYFDY

SEQ ID NO: 29 - protein, 120 aa, homo sapiens
QVQLVESGGGVVQPGRSLRLSCPASGFTFSIYAMHWVRQAPGKGLEWVAVVSNDGYNKYYADSVKGRFTISRDNSKDTLYLQMNSLRAEDTAVYYCARDGQLGRGYFDYWGQGTLVTVSS

SEQ ID NO: 30 - protein, 8 aa, homo sapiens
GFTFSIYA

SEQ ID NO: 31 - protein, 8 aa, homo sapiens
VSNDGYNK

SEQ ID NO: 32 - protein, 13 aa, homo sapiens
ARDGQLGRGYFDY

SEQ ID NO: 33 - protein, 118 aa, homo sapiens
QVQLVQSGAEVRKPGSSVKVSCKASGGSFNNYPIFWVRQAPGQGFEWMGRIIPILGITAYAQKFQGRVTITADKSTSTAYMELNSLRSEDTAVYYCAGGDDLDAFDIWGQGTMVSVSS

SEQ ID NO: 34 - protein, 8 aa, homo sapiens
GGSFNNYP

SEQ ID NO: 35 - protein, 8 aa, homo sapiens
IIPILGIT

SEQ ID NO: 36 - protein, 11 aa, homo sapiens
AGGDDLDAFDI

SEQ ID NO: 37 - protein, 120 aa, homo sapiens
QVQLVESGGGVVQPGRSLRLSCAGSGFTFNRYAMYWVRQAPGKGLDWVAVISNDGINKYYADSVKGRFTISRDNSKNTLYLQMNSLRAEDTAVYYCARDHTMVRGAFDYWGQGTLVTVSS

SEQ ID NO: 38 - protein, 8 aa, homo sapiens
GFTFNRYA

SEQ ID NO: 39 - protein, 8 aa, homo sapiens
ISNDGINK

SEQ ID NO: 40 - protein, 13 aa, homo sapiens
ARDHTMVRGAFDY

SEQ ID NO: 41 - protein, 107 aa, homo sapiens
EIVLTQSPGTLSLSPGERATLSCRASQSVSSSYLAWYQQKPGQAPRLLIYGASSRATGIPDRFSGSGSGTDFTLTISRLEPEDFAVYYCQQYGSSLTFGGGTKVEIK

SEQ ID NO: 42 - protein, 7 aa, homo sapiens
QSVSSSY

SEQ ID NO: 43 - protein, 3 aa, homo sapiens
GAS

SEQ ID NO: 44 - protein, 8 aa, homo sapiens
QQYGSSLT

SEQ ID NO: 45 - protein, 107 aa, homo sapiens
DIQMTQSPPSLSASAGDRVTITCRASQGISSRLAWYQQKPEKAPKSLIYAASSLQSGVPSRFSGSGSGTDFTLTISSLQPEDFATYYCQQYNSYPYTFGQGTKLEIK

SEQ ID NO: 46 - protein, 6 aa, homo sapiens
QGISSR

SEQ ID NO: 47 - protein, 3 aa, homo sapiens
AAS

SEQ ID NO: 48 - protein, 9 aa, homo sapiens
QQYNSYPYT

SEQ ID NO: 49 - protein, 108 aa, homo sapiens
EIVLTQSPGTLSLSPGERATLSCRASQSVRSSYLAWYQQKPGQAPRLLIYGASSRATGIPDRFSGSGSGTDFTLTISRLEPEDFAVYYCQQYGSSPRTFGQGTKVEIK

SEQ ID NO: 50 - protein, 7 aa, homo sapiens
QSVRSSY

SEQ ID NO: 51 - protein, 3 aa, homo sapiens
GAS

SEQ ID NO: 52 - protein, 9 aa, homo sapiens
QQYGSSPRT

SEQ ID NO: 53 - protein, 108 aa, homo sapiens
EIVLTQSPGTLSLSPGERATLSCRASQSVGSSSLAWYQQKPGQAPRLLIYGASSRATGIPDRFSGSGSGTDFTLTISRLEPEDFAVYYCQQYGSSPRTFGQGTKVEIK

SEQ ID NO: 54 - protein, 7 aa, homo sapiens
QSVGSSS

SEQ ID NO: 55 - protein, 3 aa, homo sapiens
GAS

SEQ ID NO: 56 - protein, 9 aa, homo sapiens
QQYGSSPRT

SEQ ID NO: 57 - protein, 107 aa, homo sapiens
DIQMTQSPSSLSASVGDRVTITCRASQGISSRLAWYQQKPEKAPKSLIYAASSLQSGVPSRFSGSGSGTDFTLTISSLQPEDFATYYCQQYNSYPYTFGQGTKLEIK

SEQ ID NO: 58 - protein, 6 aa, homo sapiens
QGISSR

SEQ ID NO: 59 - protein, 3 aa, homo sapiens
AAS

SEQ ID NO: 60 - protein, 9 aa, homo sapiens
QQYNSYPYT

SEQ ID NO: 61 - protein, 108 aa, homo sapiens
DIQMTQSPSSLSASVGDRVTITCRASQGISSWLAWYQQKPEKAPKSLIYAASSLQSGVPSRFSGSGSGTDFTLTISSLQPEDFATYYCQQYNSYPLYTFGQGTKLEIK

SEQ ID NO: 62 - protein, 6 aa, homo sapiens
QGISSW

SEQ ID NO: 63 - protein, 3 aa, homo sapiens
AAS

SEQ ID NO: 64 - protein, 10 aa, homo sapiens
QQYNSYPLYT

SEQ ID NO: 65 - protein, 107 aa, homo sapiens
EIVLTQSPATLSLSPGERATLSCRASQSVSSYLAWYQQKPGQAPRLLIYDASNRATGIPARFSGSGSGTDFTLTISSLEPEDFAVYYCQQRSNWPLTFGGGTKVEIK

SEQ ID NO: 66 - protein, 6 aa, homo sapiens
QSVSSY

SEQ ID NO: 67 - protein, 3 aa, homo sapiens
DAS

SEQ ID NO: 68 - protein, 9 aa, homo sapiens
QQRSNWPLT

SEQ ID NO: 69 - protein, 107 aa, homo sapiens
EIVLTQSPATLSLSPGERAILSCRASQSVSSYLAWYQQKPGQAPRLLIYDASNRATGIPARFSGSGSGTDFTLTISSLEPEDFAVYYCQQRSNWPLTFGGGTKVEIK

SEQ ID NO: 70 - protein, 6 aa, homo sapiens
QSVSSY

SEQ ID NO: 71 - protein, 3 aa, homo sapiens
DAS

SEQ ID NO: 72 - protein, 9 aa, homo sapiens
QQRSNWPLT

SEQ ID NO: 73 - protein, 107 aa, homo sapiens
DIQMTQSPSSLSASVGDRVTITCRASQGISSWLAWYQQKPEKAPKSLIYAASSLQSGVPSRFSGSGSGTDFTLTISSLQPEDFATYYCQQYNSYPYTFGQGTKLEIK

SEQ ID NO: 74 - protein, 6 aa, homo sapiens
QGISSW

SEQ ID NO: 75 - protein, 3 aa, homo sapiens
AAS

SEQ ID NO: 76 - protein, 9 aa, homo sapiens
QQYNSYPYT

SEQ ID NO: 77 - protein, 107 aa, homo sapiens; identical to SEQ ID NO: 65

SEQ ID NO: 78 - protein, 6 aa, homo sapiens
QSVSSY

SEQ ID NO: 79 - protein, 3 aa, homo sapiens
DAS

SEQ ID NO: 80 - protein, 9 aa, homo sapiens
QQRSNWPLT